European Patent Application EP 4 442 706 A2, published October 9, 2024. Title: CANINE ANTIBODY LIBRARIES. Applicant: Adivo GmbH. The sequence listing filed with the application follows.

SEQUENCE LISTING (47 sequences)

SEQ ID NO: 1 - protein, 96 aa, synthetic construct
  REGION 1..96: note = source = /note="Description of Artificial Sequence: Synthetic polypeptide"
EVQLVESGGDLVKPAGSLRLSCVASGFTFSSYSMSWVRQAPEKGLQLVAGINSGGSSTYYTDAVKGRFTISRDNAKNTVYLQMNSLRAEDTAMYYC

SEQ ID NO: 2 - protein, 96 aa, synthetic construct
  REGION 1..96: note = source = /note="Description of Artificial Sequence: Synthetic polypeptide"
EVQLVESGGDLVKPGGTLRLSCVASGFTFSSYDMSWVRQSPGKGLQWVAVIWNDGSSTYYADAVKGRFTISRDNAKNTLYLQMNSLRAEDTAVYYC

SEQ ID NO: 3 - protein, 96 aa, synthetic construct
  REGION 1..96: note = source = /note="Description of Artificial Sequence: Synthetic polypeptide"
EVQLVESGGNLVKPGGSLRLSCVASGLTFYSYAIYWVHEAPGKGLQWVAAITTDGSSTYYTDAVKGRFTISRDNAKNTLYLQMNSLRAEDMPVYYC

SEQ ID NO: 4 - protein, 96 aa, synthetic construct
  REGION 1..96: note = source = /note="Description of Artificial Sequence: Synthetic polypeptide"
EVQLVESGGDLVKPGGSLRLSCVASGFTFSNYEMYWVRQAPGKGLEWVARIYESGSTTYYAEAVKGRFTISRDNAKNMAYLQMNSLRAEDTAVYYC

SEQ ID NO: 5 - protein, 96 aa, synthetic construct
  REGION 1..96: note = source = /note="Description of Artificial Sequence: Synthetic polypeptide"
EVQLVQSGAEVKKPGASVKVSCKTSGYTFINYYMIWVRQAPGAGLDWMGQIDPEDGATSYAQKFQGRVTLTADTSTSTAYMELSSLRAGDIAVYYC

SEQ ID NO: 6 - protein, 96 aa, synthetic construct
  REGION 1..96: note = source = /note="Description of Artificial Sequence: Synthetic polypeptide"
EVQLVESGGDLVKPAGSLRLSCVASGFTFSSYSMSWVRQAPEKGLQLVAGISSGGSSTYYTDAVKGRFTISRDNAKNTVYLQMNSLRAEDTAMYYC

SEQ ID NO: 7 - protein, 96 aa, synthetic construct
  REGION 1..96: note = source = /note="Description of Artificial Sequence: Synthetic polypeptide"
EVQLVESGGDLVKPGGTLRLSCVASGFTFSSYDMSWVRQSPGKGLQWVAVIWNEGSSTYYADAVKGRFTISRDNAKNTLYLQMNSLRAEDTAVYYC

SEQ ID NO: 8 - protein, 96 aa, synthetic construct
  REGION 1..96: note = source = /note="Description of Artificial Sequence: Synthetic polypeptide"
EVQLVESGGNLVKPGGSLRLSCVASGLTFYSYAIYWVHEAPGKGLQWVAAITTGGSSTYYTDAVKGRFTISRDNAKNTLYLQMNSLRAEDMPVYYC

SEQ ID NO: 9 - protein, 96 aa, synthetic construct; identical to SEQ ID NO: 4
  REGION 1..96: note = source = /note="Description of Artificial Sequence: Synthetic polypeptide"

SEQ ID NO: 10 - protein, 96 aa, synthetic construct
  REGION 1..96: note = source = /note="Description of Artificial Sequence: Synthetic polypeptide"
EVQLVQSGAEVKKPGASVKVSCKTSGYTFINYYMIWVRQAPGAGLDWMGQIDPEGGATSYAQKFQGRVTLTADTSTSTAYMELSSLRAGDIAVYYC

SEQ ID NO: 11 - protein, 93 aa, synthetic construct
  REGION 1..93: note = source = /note="Description of Artificial Sequence: Synthetic polypeptide"
DIVMTQTPLSLSVSPGEPASISCKASQSLLHSNGNTYLYWFRQKPGQSPQRLIYKVSNRDPGVPDRFSGSGSGTDFTLRISRVEAEDAGVYYC

SEQ ID NO: 12 - protein, 88 aa, synthetic construct
  REGION 1..88: note = source = /note="Description of Artificial Sequence: Synthetic polypeptide"
EIVMTQSPASLSLSQEEKVTITCRASQSVSSYLAWYQQKPGQAPKLLIYGTSNRATGVPSRFSGSGSGTDFSFTISSLEPEDVAVYYC

SEQ ID NO: 13 - protein, 87 aa, synthetic construct
  REGION 1..87: note = source = /note="Description of Artificial Sequence: Synthetic polypeptide"
SYVLTQLPSVSVTLRQTARITCGGDSIGSKNVYWYQQKLGQAPVLIIYDDSSRPSGIPERFSGANSGNTATLTISGALAEDEADYYC

SEQ ID NO: 14 - protein, 90 aa, synthetic construct
  REGION 1..90: note = source = /note="Description of Artificial Sequence: Synthetic polypeptide"
QTVVTQEPSLSVSPGGTVTLTCGLSSGSVSTSNYPGWYQQTLGRAPRTIIYRTSSRPSGVPNRFSGSISGNKAALTITGAQPEDEADYYC

SEQ ID NO: 15 - protein, 90 aa, synthetic construct
  REGION 1..90: note = source = /note="Description of Artificial Sequence: Synthetic polypeptide"
QSVLTQPASVSGSLGQRVTISCTGSSSNVGYGNYVGWYQQLPGTGPRTLIYRSSSRPSGVPDRFSGSRSGSTATLTISGLQAEDEADYYC

SEQ ID NO: 16 - protein, 89 aa, synthetic construct
  REGION 1..89: note = source = /note="Description of Artificial Sequence: Synthetic polypeptide"
QSVLTQPASVSGSLGQRVTISCTGSSSNIGRGYVGWYQQLPGTGPRTLIYGNSNRPSGVPDRFSGSRSGSTATLTISGLQAEDEADYYC

SEQ ID NO: 17 - protein, 93 aa, synthetic construct
  REGION 1..93: note = source = /note="Description of Artificial Sequence: Synthetic polypeptide"
DIVMTQTPLSLSVSPGEPASISCKASQSLLHSSGNTYLYWFRQKPGQSPQRLIYKVSNRDPGVPDRFSGSGSGTDFTLRISRVEAEDAGVYYC

SEQ ID NO: 18 - protein, 89 aa, synthetic construct
  REGION 1..89: note = source = /note="Description of Artificial Sequence: Synthetic polypeptide"
QSVLTQPASVSGSLGQRVTISCTGSSSNIGRGYVGWYQQLPGTGPRTLIYGISNRPSGVPDRFSGSRSGSTATLTISGLQAEDEADYYC

SEQ ID NO: 19 - DNA, 288 bp, synthetic construct
  misc_feature 1..288: note = source = /note="Description of Artificial Sequence: Synthetic polynucleotide"
  source 1..288: mol_type = other DNA
gaagtgcaattggtggaaagcggtggcgatctggtgaaaccagccggcagcctgcgcctgagctgcgtggccagcggctttacctttagcagctatagcatgagctgggttcgccaggccccggaaaaaggcctgcagctggtggccggcattaatagcggcggcagcagcacctattataccgatgccgtgaaaggccgctttaccattagccgcgataacgccaaaaacaccgtgtacctgcagatgaacagcctgcgggccgaagataccgccatgtattattgc

SEQ ID NO: 20 - DNA, 288 bp, synthetic construct
  misc_feature 1..288: note = source = /note="Description of Artificial Sequence: Synthetic polynucleotide"
  source 1..288: mol_type = other DNA
gaagtgcaattggttgaaagcggtggtgatctggttaaaccgggtggcaccctgcgtctgagctgtgttgcaagcggttttacctttagcagctatgatatgagctgggtgcgccagagtccgggtaaaggtctgcagtgggttgcagttatttggaatgatggtagcagcacctattatgcagatgcagttaaagggcgttttaccattagccgtgataatgccaaaaataccctgtatctgcagatgaatagcctgcgtgcagaggataccgcagtgtattattgc

SEQ ID NO: 21 - DNA, 288 bp, synthetic construct
  misc_feature 1..288: note = source = /note="Description of Artificial Sequence: Synthetic polynucleotide"
  source 1..288: mol_type = other DNA
gaagtgcaattggttgaaagcggtggtaatctggttaaaccgggtggtagcctgcgtctgagctgtgttgcaagcggtctgaccttttatagctatgcaatttattgggtgcacgaagcaccgggaaaaggtctgcagtgggttgcagcaattaccaccgatggcagcagcacctattacaccgatgcagttaaagggcgttttaccattagccgtgataatgccaaaaataccctgtatctgcagatgaatagcctgcgtgcagaggatatgccggtgtattattgc

SEQ ID NO: 22 - DNA, 288 bp, synthetic construct
  misc_feature 1..288: note = source = /note="Description of Artificial Sequence: Synthetic polynucleotide"
  source 1..288: mol_type = other DNA
gaagtgcaattggttgaaagcggtggtgatctggttaaaccgggtggtagcctgcgtctgagctgtgttgcaagcggttttacctttagcaactatgaaatgtattgggtgcggcaggcaccgggtaaaggtctggaatgggttgcacgcatttatgaaagcggtagcaccacctattatgcagaagcagttaaagggcgttttaccattagccgtgataacgccaaaaatatggcatatctgcagatgaatagcctgcgtgcagaggataccgcagtgtattattgc

SEQ ID NO: 23 - DNA, 288 bp, synthetic construct
  misc_feature 1..288: note = source = /note="Description of Artificial Sequence: Synthetic polynucleotide"
  source 1..288: mol_type = other DNA
gaagtgcaattggttcagagcggtgccgaagttaaaaaaccgggtgcaagcgttaaagttagctgtaaaaccagcggctataccttcatcaactattatatgatttgggtgcgccaggcaccgggtgcaggtctggattggatgggtcagattgatccggaagaaggtgcaaccagctatgcacagaaatttcagggtcgtgttaccctgaccgcagataccagcaccagcaccgcatatatggaactgagcagcctgcgtgccggtgatattgcagtgtattattgc

SEQ ID NO: 24 - DNA, 288 bp, synthetic construct
  misc_feature 1..288: note = source = /note="Description of Artificial Sequence: Synthetic polynucleotide"
  source 1..288: mol_type = other DNA
gaagtgcaattggtggaaagcggtggcgatctggtgaaaccagccggcagcctgcgcctgagctgcgtggccagcggctttacctttagcagctatagcatgagctgggttcgccaggccccggaaaaaggcctgcagctggtggccggcattagcagcggcggcagcagcacctattataccgatgccgtgaaaggccgctttaccattagccgcgataacgccaaaaacaccgtgtacctgcagatgaacagcctgcgggccgaagataccgccatgtattattgc

SEQ ID NO: 25 - DNA, 288 bp, synthetic construct
  misc_feature 1..288: note = source = /note="Description of Artificial Sequence: Synthetic polynucleotide"
  source 1..288: mol_type = other DNA
gaagtgcaattggttgaaagcggtggtgatctggttaaaccgggtggcaccctgcgtctgagctgtgttgcaagcggttttacctttagcagctatgatatgagctgggtgcgccagagtccgggtaaaggtctgcagtgggttgcagttatttggaatgaaggtagcagcacctattatgcagatgcagttaaagggcgttttaccattagccgtgataatgccaaaaataccctgtatctgcagatgaatagcctgcgtgcagaggataccgcagtgtattattgc

SEQ ID NO: 26 - DNA, 288 bp, synthetic construct
  misc_feature 1..288: note = source = /note="Description of Artificial Sequence: Synthetic polynucleotide"
  source 1..288: mol_type = other DNA
gaagtgcaattggttgaaagcggtggtaatctggttaaaccgggtggtagcctgcgtctgagctgtgttgcaagcggtctgaccttttatagctatgcaatttattgggtgcacgaagcaccgggaaaaggtctgcagtgggttgcagcaattaccaccggtggcagcagcacctattacaccgatgcagttaaagggcgttttaccattagccgtgataatgccaaaaataccctgtatctgcagatgaatagcctgcgtgcagaggatatgccggtgtattattgc

SEQ ID NO: 27 - DNA, 288 bp, synthetic construct; identical to SEQ ID NO: 22
  misc_feature 1..288: note = source = /note="Description of Artificial Sequence: Synthetic polynucleotide"
  source 1..288: mol_type = other DNA

SEQ ID NO: 28 - DNA, 288 bp, synthetic construct
  misc_feature 1..288: note = source = /note="Description of Artificial Sequence: Synthetic polynucleotide"
  source 1..288: mol_type = other DNA
gaagtgcaattggttcagagcggtgccgaagttaaaaaaccgggtgcaagcgttaaagttagctgtaaaaccagcggctataccttcatcaactattatatgatttgggtgcgccaggcaccgggtgcaggtctggattggatgggtcagattgatccggaaggtggtgcaaccagctatgcacagaaatttcagggtcgtgttaccctgaccgcagataccagcaccagcaccgcatatatggaactgagcagcctgcgtgccggtgatattgcagtgtattattgc

SEQ ID NO: 29 - DNA, 279 bp, synthetic construct
  misc_feature 1..279: note = source = /note="Description of Artificial Sequence: Synthetic polynucleotide"
  source 1..279: mol_type = other DNA
gatattgtgatgacccagaccccactgagcctgagcgtgagcccaggcgaaccagccagcattagctgcaaagccagccagagcctgctgcatagcaatggcaacacctatctgtattggtttcgccagaaaccaggccagagcccacagcgcctgatctataaagtgagcaaccgcgatccaggcgtgccggatcgctttagcggcagcggtagcggcaccgattttaccctgcgcattagtcgcgtggaagccgaagacgcaggcgtgtattattgc

SEQ ID NO: 30 - DNA, 264 bp, synthetic construct
  misc_feature 1..264: note = source = /note="Description of Artificial Sequence: Synthetic polynucleotide"
  source 1..264: mol_type = other DNA
gaaattgttatgacccagagtccggcaagcctgagcctgagccaagaagaaaaagttaccattacctgtcgtgcaagccagagcgttagcagctatctggcatggtatcagcagaaaccgggtcaggcaccgaaactgctgatttatggcaccagcaatcgtgcaaccggtgttccgagccgttttagcggtagcggtagtggcaccgattttagctttaccattagcagcctggaaccggaagacgtggccgtgtattattgc

SEQ ID NO: 31 - DNA, 261 bp, synthetic construct
  misc_feature 1..261: note = source = /note="Description of Artificial Sequence: Synthetic polynucleotide"
  source 1..261: mol_type = other DNA
agctatgtgctgacccagctgccgagcgtgagcgtgaccctgcgccagaccgcacgcattacctgcggtggcgatagcattggcagcaaaaacgtgtattggtatcagcagaaactgggccaggcaccggtgctgattatctatgatgatagcagtcgcccaagcggcattccggaacgctttagcggtgccaacagcggcaacaccgccaccctgaccattagcggtgccctggccgaagacgaagccgattattactgc

SEQ ID NO: 32 - DNA, 270 bp, synthetic construct
  misc_feature 1..270: note = source = /note="Description of Artificial Sequence: Synthetic polynucleotide"
  source 1..270: mol_type = other DNA
cagaccgttgttacccaagaaccgagcctgagcgttagtccgggtggcaccgttaccctgacctgtggtctgagcagcggtagcgttagcaccagcaattatccagggtggtatcagcagaccctgggtcgtgcaccgcgtaccattatctatcgtaccagcagccgtccgagcggtgttccgaatcgttttagcggtagcattagcggtaataaagcagcactgaccattaccggtgcacagccggaagacgaagccgattattactgc

SEQ ID NO: 33 - DNA, 270 bp, synthetic construct
  misc_feature 1..270: note = source = /note="Description of Artificial Sequence: Synthetic polynucleotide"
  source 1..270: mol_type = other DNA
cagagcgttctgacccagcctgcaagcgttagcggtagcctgggtcagcgtgttaccattagctgtaccggtagtagtagcaatgttggttatggtaattatgttggttggtatcagcagctgcctggcaccggtccgcgtaccctgatttatcgtagcagcagccgtccgagcggtgttccggatcgttttagcggtagtcgtagcggtagcaccgcaaccctgaccattagcggtctgcaggcagaagacgaagccgattattactgc

SEQ ID NO: 34 - DNA, 267 bp, synthetic construct
  misc_feature 1..267: note = source = /note="Description of Artificial Sequence: Synthetic polynucleotide"
  source 1..267: mol_type = other DNA
cagagcgttctgacccagcctgcaagcgttagcggtagcctgggtcagcgtgttaccattagctgtaccggtagtagcagcaatattggtcgtggttatgttggttggtatcagcagctgcctggcaccggtccgcgtaccctgatttatggtaatagcaatcgtccgagcggtgttccggatcgttttagcggtagtcgtagcggtagcaccgcaaccctgaccattagcggtctgcaggcagaagacgaagccgattattactgc

SEQ ID NO: 35 - DNA, 279 bp, synthetic construct
  misc_feature 1..279: note = source = /note="Description of Artificial Sequence: Synthetic polynucleotide"
  source 1..279: mol_type = other DNA
gatattgtgatgacccagaccccactgagcctgagcgtgagcccaggcgaaccagccagcattagctgcaaagccagccagagcctgctgcatagcagcggcaacacctatctgtattggtttcgccagaaaccaggccagagcccacagcgcctgatctataaagtgagcaaccgcgatccaggcgtgccggatcgctttagcggcagcggtagcggcaccgattttaccctgcgcattagtcgcgtggaagccgaagacgcaggcgtgtattattgc

SEQ ID NO: 36 - DNA, 267 bp, synthetic construct
  misc_feature 1..267: note = source = /note="Description of Artificial Sequence: Synthetic polynucleotide"
  source 1..267: mol_type = other DNA
cagagcgttctgacccagcctgcaagcgttagcggtagcctgggtcagcgtgttaccattagctgtaccggtagtagcagcaatattggtcgtggttatgttggttggtatcagcagctgcctggcaccggtccgcgtaccctgatttatggtattagcaatcgtccgagcggtgttccggatcgttttagcggtagtcgtagcggtagcaccgcaaccctgaccattagcggtctgcaggcagaagacgaagccgattattactgc

SEQ ID NO: 37 - protein, 11 aa, synthetic construct
  REGION 1..11: note = source = /note="Description of Artificial Sequence: Synthetic peptide"
WGQGTLVTVSS

SEQ ID NO: 38 - protein, 10 aa, synthetic construct
  REGION 1..10: note = source = /note="Description of Artificial Sequence: Synthetic peptide"
FGAGTKVELK

SEQ ID NO: 39 - protein, 10 aa, synthetic construct
  REGION 1..10: note = source = /note="Description of Artificial Sequence: Synthetic peptide"
FGGGTQLTVL

SEQ ID NO: 40 - DNA, 33 bp, synthetic construct
  misc_feature 1..33: note = source = /note="Description of Artificial Sequence: Synthetic oligonucleotide"
  source 1..33: mol_type = other DNA
tggggccagggcaccctggttaccgtctcgagc

SEQ ID NO: 41 - DNA, 30 bp, synthetic construct
  misc_feature 1..30: note = source = /note="Description of Artificial Sequence: Synthetic oligonucleotide"
  source 1..30: mol_type = other DNA
tttggcgcaggtaccaaagtggaactgaaa

SEQ ID NO: 42 - DNA, 30 bp, synthetic construct
  misc_feature 1..30: note = source = /note="Description of Artificial Sequence: Synthetic oligonucleotide"
  source 1..30: mol_type = other DNA
tttggcggtggtacccagctgaccgtgctg

SEQ ID NO: 43 - protein, 11 aa, synthetic construct
  REGION 1..11: note = source = /note="Description of Artificial Sequence: Synthetic peptide"
WGGDGFYAMDY

SEQ ID NO: 44 - protein, 9 aa, synthetic construct
  REGION 1..9: note = source = /note="Description of Artificial Sequence: Synthetic peptide"
QQHYTTPPT

SEQ ID NO: 45 - protein, 11 aa, synthetic construct
  REGION 1..11: note = source = /note="Description of Artificial Sequence: Synthetic peptide"
QSYDSSLSGVV

SEQ ID NO: 46 - protein, 4 aa, synthetic construct
  REGION 1..4: note = source = /note="Description of Artificial Sequence: Synthetic peptide"
EVQL

SEQ ID NO: 47 - protein, 6 aa, synthetic construct
  REGION 1..6: note = source = /note="Description of Artificial Sequence: Synthetic 6xHis tag"
HHHHHH